European Patent Specification EP 3 526 323 B1, published March 29, 2023. Title: ENGINEERED NUCLEASES SPECIFIC FOR RECOGNITION SEQUENCES IN THE HEPATITIS B VIRUS GENOME. Applicant: Precision Biosciences, Inc. The sequence listing filed with the application follows.

SEQUENCE LISTING (86 sequences)

SEQ ID NO: 1 - protein, 163 aa, Chlamydomonas reinhardtii
  wild-type I-CreI meganuclease (1)..(163)
MNTKYNKEFLLYLAGFVDGDGSIIAQIKPNQSYKFKHQLSLAFQVTQKTQRRWFLDKLVDEIGVGYVRDRGSVSDYILSEIKPLHNFLTQLQPFLKLKQKQANLVLKIIWRLPSAKESPDKFLEVCTWVDQIAALNDSKTRKTTSETVRAVLDSLSEKKKSSP

SEQ ID NO: 2 - protein, 9 aa, Chlamydomonas reinhardtii
  LAGLIDADG (1)..(9)
LAGLIDADG

SEQ ID NO: 3 - DNA, 3221 bp, Hepatitis B virus
  HBV genotype A (1)..(3221)
ttccactgccttccaccaagctctgcaggatcccagagtcaggggtctgtattttcctgctggtggctccagttcaggaacagtaaaccctgctccgaatattgcctctcacatctcgtcaatctccgcgaggactggggaccctgtggcgaacatggagaacatcacatcaggattcctaggacccctgctcgtgttacaggcggggtttttcttgttgacaagaatcctcacaataccgcagagtctagactcgtggtggacttctctcaattttctagggggatcacccgtgtgtcttggccaaaattcgcagtccccaacctccaatcactcaccaacctcctgtcctccaatttgtcctggttatcgctggatgtgtctgcggcgttttatcatattcctcttcatcctgctgctatgcctcatcttcttattggttcttctggattatcaaggtatgttgcccgtttgtcctctaattccaggatcaacaacaaccagtacgggaccatgcaaaacctgcacgactcctgctcaaggcaactctatgtttccctcatgttgctgtacaaaacctacggatggaaattgcacctgtattcccatcccatcgtcctgggctttcgcaaaatacctatgggagtgggcctcagtccgtttctcttggctcagtttactagtgccatttgttcagtggttcgtagggctttcccccactgtttggctttcagctatatggatgatgtggtattgggggccaagtctgtacagcatcgtgagtccctttataccgctgttaccaattttcttttgtctctgggtatacatttaaaccctaacaaaacaaaaagatggggttattccctaaacttcatgggttacataattggaagttggggaactttgccacaggatcatattgtacaaaagatcaaacactgttttagaaaacttcctgttaacaggcctattgattggaaagtatgtcaaagaattgtgggtcttttgggctttgctgctccatttacacaatgtggatatcctgccttaatgcctttgtatgcatgtatacaagctaaacaggctttcactttctcgccaacttacaaggcctttctaagtaaacagtacatgaacctttaccccgttgctcggcaacggcctggtctgtgccaagtgtttgctgacgcaacccccactggctggggcttggccataggccatcagcgcatgcgtggaacctttgtggctcctctgccgatccatactgcggaactcctagccgcttgttttgctcgcagccggtctggagcaaagctcatcggaactgacaattctgtcgtcctctcgcggaaatatacatcgtttccatggctgctaggctgtgctgccaactggatccttcgcggaacgtcctttgtctacgtcccgtcggcgctgaatcccgcggacgacccctctcggggccgcttgggactctctcgtccccttctccgtctgccgttccagccgaccacggggcgcacctctctttacgcggtctccccgtctgtgccttctcatctgccggtccgtgtgcacttcgcttcacctctgcacgttgcatggagaccaccgtgaacgcccatcagatcctgcccaaggtcttacataagaggactcttggactcccagcaatgtcaacgaccgaccttgaggcctacttcaaagactgtgtgtttaaggactgggaggagctgggggaggagattaggttaaaggtctttgtattaggaggctgtaggcataaattggtctgcgcaccagcaccatgcaactttttcacctctgcctaatcatctcttgtacatgtcccactgttcaagcctccaagctgtgccttgggtggctttggggcatggacattgacccttataaagaatttggagctactgtggagttactctcgtttttgccttctgacttctttccttccgtcagagatctcctagacaccgcctcagctctgtatcgagaagccttagagtctcctgagcattgctcacctcaccatactgcactcaggcaagccattctctgctggggggaattgatgactctagctacctgggtgggtaataatttggaagatccagcatccagggatctagtagtcaattatgttaatactaacatgggtttaaagatcaggcaactattgtggtttcatatatcttgccttacttttggaagagagactgtacttgaatatttggtctctttcggagtgtggattcgcactcctccagcctatagaccaccaaatgcccctatcttatcaacaattccggaaactactgttgttagacgacgggaccgaggcaggtcccctagaagaagaactccctcgcctcgcagacgcagatctcaatcgccgcgtcgcagaagatctcaatctcgggaatctcaatgttagtattccttggactcataaggtgggaaactttacggggctttattcctctacagtacctatctttaatcctgaatggcaaactccttcctttcctaagattcatttacaagaggacattattaataggtgtcaacaatttgtgggccctctcactgtaaatgaaaagagaagattgaaattaattatgcctgctagattctatcctacccacactaaatatttgcccttagacaaaggaattaaaccttattatccagatcaggtagttaatcattacttccaaaccagacattatttacatactctttggaaggctggtattctatataagagggaaaccacacgtagcgcatcattttgcgggtcaccatattcttgggaacaagagctacagcatgggaggttggtcatcaaaacctcgcaaaggcatggggacgaatctttctgttcccaaccctctgggattctttcccgatcatcagttggaccctgcattcggagccaactcaaacaatccagattgggacttcaaccccatcaaggaccactggccaacagccaaccaggtaggagtgggagcattcgggccagggctcacccctccacacggcggtattttgggggggagccctcaggctcagggcatattgaccacagtgtcaacaattcctcctcctgcctccaccaatcggcagtcaggaaggcagcctactcccatctctccacctctaagagacagtcatcctcaggccatgcagtggaa

SEQ ID NO: 4 - DNA, 3214 bp, Hepatitis B virus
  HBV genotype B (1)..(3214)
tccaccactttccaccaaactcttcaagatcccagagtcagggccctgtactttcctgctggtggctccagttcaggaacagtgagccctgctcagactactgtctctgccatatcgtcaatcttatcgaagactggggaccctgtaccgaacatggagaacatcgcatcaggactcctaggacccctgctcgtgttacaggcggggtttttcttgttgacaaaaatcctcacaataccacagagtctagactcgtggtggacttctctcaattttctagggggaamacccgtgtgtcttggccaaaattcgcagtcccaaatctccagtcactcacyaacctgttgtcctccaatttgtcctggttatcgctggatgtgtctgcggcgttttatcatcttcctytgcatcctgctgctatgcctcatcttcttgttggttcttctggactatcraggtatgttgcccgtttgtcctcwamttccaggatcawcaacaaccagcaccggaccatgcaaaacctgcacgactcctgctcaaggaacctctatryktccctcatgttgctgtacaaaacctacggacggaaactgcacctgtattcccatcccatcatcttgggctttcgcaaaatacctatgggagtsggcctcagyccgtttctcttggctcagtttactagcgccatttgttcagtggttcgtagggctttcccccactgtctggctttcagttatatggatgatgtggtattgggggccaagtctgtacaacatcttgagtccctttatgccgctgttaccaatttycttttgtctttgggtatacayttgaaccctcacaaaacaaaaagatggggatattcccttaacttcatgggatatgtaattgggtgttggggcacattgccacaggaacatattgtacaaaaaatcaaaatgtgttttmggaaacttcctgtaaacagacctattgattggaaagtatgtcaacgaattgtgggtcttttggggtttgccgcccctttcacgcaatgtggatatcctgctttratgcctttatatgcatgtatacaagcaaaacaggcttttactttctcgccaacttacaaggcctttctaagtaaacagtatctgaacctttaccccgttactcggcaacggtctggtctgtgccaagtgtttgctgacgcaacccccactggttggggcttggccataggccwtcagcgcatgcgtggaacctttgtgtctcctctgccgatccatactgcggaactcctagccgcttgttttgctcgcagcaggtctggggcaaaactcatcgggactgacaattctgtcgtgctctcccgcaagtatacatcgttcccatggctgctaggctgtgctgccaactggatcctgcgcgggacgtcctttgtttacgtcccgtcggcgctgaatcccgcggacgacccctcccggggccgcttggggctctaccgcccgcttctccgcctgttgtaccgtccgaccacggggcgcacctctctttacgcggactccccgtctgtgccttctcatctrccggaccgtgtgcacttcgcttcacctctgcacgtcgcatggagaccaccgtgaacgcccaccggaacctgcccaaggtcttgcataagaggactcttggactttccgcaatgtcaacgaccgaccttgaggcatacttcaaagactgtgtgtttamtgagtgggaggagttgggggaggagaktaggttaaaggtctttgtactaggaggctgtaggcataaattggtgtgttcaccagcaccatgcaactttttcacctctgcctaatcatctcwtgttcatgtcctactgttcaagcctccaagctgtgccttgggtggctttagggcatggacattgacccgtataaagaatttggagcttctgtggagttactctcttttttgcctmmtgacttctttccttctattcgagatctcctcgacaccgcctctgctttgtatcgggaggccttagagtctccggaacattgttcacctcaccatacggcactcaggcaagctattctgtgttggggtgagttgatgaatctagccacctgggtgggaagtaatttggaagatccagcatccagggaattagtmgttagctatgtcaacgttaatatgggcmtaaaaatcagacaactattgtggtttcacatttcctgtcttacttttgggaragamactgttcttgaatatttggtgtcttttggagtgtggattcgcactcctcctgcatatagaccaycaaatgcccctatcttatcaacacttccggaaactactgttgttagacgaagaggcaggtcccctagaagaagaactccctcgcctcgcagacgaaggtctcaatcgccgcgtcgcagaagatctcaatctcgggaatctcaatgttagtattccttggacacataaggtgggaaactttacggggctttattcttctacggtaccttgctttaatcctaawtggcaaactccttcttttcctgacattcatttgcaggaggacattgttgatagatgtaagcamtttgtggggccccttacagtaaatgaaaacaggagactaaaattaattatgcctgctaggttttatcccaatgttaccaaatatttgcccttagataaagggatcaaaccttattatccagagcatgtagttaatcattacttccagacgagacattatttacayactctttggaaggcgggtatcytatataaaagagagtccacacgtagcgcctcattttgcggatcaccatattcttgggaacaagatctacagcatgggaggttggtcttccaaacctcgaaaaggcatggggacaaatctttctgtccccaatcccctgggattcttcccmgatcatcagttggaccctgcattcaaagccaactcasaaaatccagattgggacctcaacccgcacaaggacaactggccggacgccaacaaggtgggagtgggagcattcgggccagggttcatccctccccatgggggactgttggggtggarccctcaggctcagggcatactcacaactgtgccagcagctcctcctcctgcctccaccaatcggcagtcaggaaggcagcctactcccttatctccacctctaagggacactcatcctcaggccatgcagtggaa

SEQ ID NO: 5 - DNA, 3214 bp, Hepatitis B virus
  HBV genotype C (1)..(3214)
tccacaacattccaccaagctctgctagatcccagagtgaggggcctatattttcctgctggtggctccagttccggaacagtaaaccctgttccgactactgcctcacccatatcgtcaatcttctcgaggactggggaccctgcaccgaacatggagagcacaacatcaggattcctaggacccctgctcgtgttacaggcggggtttttcttgttgacaagaatcctcacaataccacagagtctagactcgtggtggacttctctcaattttctagggggagcacccacgtgtcctggccaaaattcgcagtccccaacctccaatcactcaccaacctcttgtcctccaatttgtcctggctatcgctggatgtgtctgcggcgttttatcatattcctcttcatcctgctgctatgcctcatcttcttgttggttcttctggactaccaaggtatgttgcccgtttgtcctctacttccaggaacatcaactaccagcacgggaccatgcaagacctgcacgattcctgctcaaggaacctctatgtttccctcttgttgctgtacaaaaccttcggacggaaactgcacttgtattcccatcccatcatcctgggctttcgcaagattcctatgggagtgggccttagtccgtttctcctggctcagtttactagtgccatttgttcagtggttcgcagggctttcccccactgtttggctttcagttatatggatgatgtggtattgggggccaagtctgtacaacatcttgagtccctttttacctctattaccaattttcttttgtcgttgggtatacatttgaaccctaataaaaccaaacgttggggctactcccttaacttcatgggatatgtaattggaagttgggggactttaccacaggaacatattgtattaaaaatcaagcaatgttttcggaaactgcctgtaaatagacctattgattggaaagtatgtcaaagaattgtgggtcttttgggctttgctgccccttttacacaatgtggctatcctgccttgatgcctttatatgcatgtatacaatctaagcaggctttcactttctcgccaacttacaaggcctttctgtgtcaacaatacctgcacctttaccccgttgcccggcaacggtcaggtctctgccaagtgtttgctgacgcaacccccactggatggggcttggccataggccatcggcgcatgcgtggaacctttgtggctcctctgccgatccatactgcggaactcctagcagcttgttttgctcgcagccggtctggagcaaaacttatcgggactgacaactctgttgtcctctctcggaaatacacctccttcccatggctgctcgggtgtgctgccaactggatcctgcgcgggacgtcctttgtctacgtcccgtcggcgctgaatcccgcggacgacccgtctcggggccgtttgggcctctaccgtccccttcttcatctgctgttccagccgactacggggcgcacctctctttacgcggtctccccgtctgtgccttctcatctgccggaccgtgtgcacttcgcttcacctctgcacgtcgcatggagaccaccgtgaatgcccaccaggtcttgcccaagctcttacataagaggactcttggactctcagcaatgtcaacgaccgaccttgaagcatacttcaaagactgtttgtttaaggactgggaggagttgggggaggagattaggttaaaggtctttgtactaggaggctgtaggcataaattggtctgttcaccagcaccatgcaactttttcacctctgcctaatcatctcatgttcatgtcctactgttcaagcctccaagctgtgccttgggtggctttggggcatggacattgacccgtataaagaatttggagcttctgtggagttactctcttttttgccttctgacttctttccttctattcgagatctcctcgacaccgcctctgctctgtatcgggaggccttagagtctccggaacattgttcacctcaccatacagcactcaggcaagctattctctgttggggtgagttgatgaatctggccacctgggtgggaagtaatttggaagacccagcatccagggaattagtagtcagctatgtcaatgttaatatgggcctaaaaatcagacaactattgtggtttcacatttcctgtcttacttttggaagagaaactgttcttgagtatttggtgtcttttggagtgtggattcgcactcctccagcttacagaccaccaaatgcccctatcttatcaacacttccggaaactactgttgttagacgacgaggcaggtcccctagaagaagaactccctcgcctcgcagacgaaggtctcaatcgccgcgtcgcagaagatctcaatctcgggaatctcaatgttagtatcccttggactcataaggtgggaaactttactgggctttattcttctactgttcctgtctttaatcctgagtggcaaactccctcctttcctaacattcatttacaggaagacattattaatagatgtcaacaatatgtgggccctcttacagttaatgaaaaaaggagattaaaattaattatgcctgctaggttctatcctaaccttaccaaatatttgcccttggataaaggcattaaaccttattatcctgaacatgcagttaatcattacttcaaaactaggcattatttacatactctgtggaaggctggcattctatataaaagagaaactacacgcagcgcttcattttgtgggtcaccatattcttgggaacaagagctacagcatgggaggttggtcttccaaacctcgacaaggcatggggacgaatctttctgttcccaatcctctgggattctttcccgatcaccagttggaccctgcgttcggagccaactcaaacaatccagattgggacttcaaccccaacaaggatcactggccagaggcaaatcaggtaggagcgggagcattcgggccagggttcaccccaccacacggcggtcttttggggtggagccctcaggctcagggcatattgacaacagtgccagcagcgcctcctcctgcctccaccaatcggcagtcaggaagacagcctactcccatctctccacctctaagagacagtcatcctcaggccatgcagtggaa

SEQ ID NO: 6 - DNA, 3182 bp, Hepatitis B virus
  HBV genotype D (1)..(3182)
ttccacaacctttcaccaaactctgcaagatcccagagtgagaggcctgtatttccctgctggtggctccagttcaggagcagtaaaccctgttccgactactgcctctcccttatcgtcaatcttctcgaggattggggaccctgcgctgaacatggagaacatcacatcaggattcctaggaccccttctcgtgttacaggcggggtttttcttgttgacaagaatcctcacaataccgcagagtctagactcgtggtggacttctctcaattttctagggggaactaccgtgtgtcttggccaaaattcgcagtccccaacctccaatcactcaccaacctcctgtcctccaacttgtcctggttatcgctggatgtgtctgcggcgttttatcatcttcctcttcatcctgctgctatgcctcatcttcttgttggttcttctggactatcaaggtatgttgcccgtttgtcctctaattccaggatcctcaaccaccagcacgggaccatgccgaacctgcatgactactgctcaaggaacctctatgtatccctcctgttgctgtaccaaaccttcggacggaaattgcacctgtattcccatcccatcatcctgggctttcggaaaattcctatgggagtgggcctcagcccgtttctcctggctcagtttactagtgccatttgttcagtggttcgtagggctttcccccactgtttggctttcagttatatggatgatgtggtattgggggccaagtctgtacagcatcttgagtccctttttaccgctgttaccaattttcttttgtctttgggtatacatttaaaccctaacaaaacaaagagatggggttactctctgaattttatgggttatgtcattggaagttatgggtccttgccacaagaacacatcatacaaaaaatcaaagaatgttttagaaaacttcctattaacaggcctattgattggaaagtatgtcaacgaattgtgggtcttttgggttttgctgccccatttacacaatgtggttatcctgcgttaatgcccttgtatgcatgtattcaatctaagcaggctttcactttctcgccaacttacaaggcctttctgtgtaaacaatacctgaacctttaccccgttgcccggcaacggccaggtctgtgccaagtgtttgctgacgcaacccccactggctggggcttggtcatgggccatcagcgcgtgcgtggaaccttttcggctcctctgccgatccatactgcggaactcctagccgcttgttttgctcgcagcaggtctggagcaaacattatcgggactgataactctgttgtcctctcccgcaaatatacatcgtatccatggctgctaggctgtgctgccaactggatcctgcgcgggacgtcctttgtttacgtcccgtcggcgctgaatcctgcggacgacccttctcggggtcgcttgagactctctcgtccccttctccgtctgccgttccgaccgaccacggggcgcacctctctttacgcggactccccgtctgtgccttctcatctgccggaccgtgtgcacttcgcttcacctctgcacgtcgcatggagaccaccgtgaacgcccaccgaatgttgcccaaggtcttacataagaggactcttggactctctgcaatgtcaacgaccgaccttgaggcatacttcaaagactgtttgtttaaagactgggaggagttgggggaggagattagattaaaggtctttgtactaggaggctgtaggcataaattggtctgcgcaccggcgccatgcacctttttcacctctgcctaatcatctcttgttcatgtcctactgttcaagcctccaagctgtgccttgggtggctttggggcatggacatcgacccttataaagaatttggagctactgtggagttactctcgtttttgccttctgacttctttccttcagtacgagatcttctagataccgcctcagctctgtatcgggaagccttagagtctcctgagcattgttcacctcaccatactgcactcaggcaagcaattctttgctggggggaactaatgactctagctacctgggtgggtgttaatttggaagatccagcatctagagacctagtagtcagttatgtcaacactaatatgggcctaaagttcaggcaactcttgtggtttcacatttcttgtctcacttttggaagagaaaccgttatagagtatttggtgtctttcggagtgtggattcgcactcctccagcttatagaccaccaaatgcccctatcctatcaacacttccggaaactactgttgttagacgacgaggcaggtcccctagaagaagaactccctcgcctcgcagacgaaggtctcaatcgccgcgtcgcagaagatctcaatctcgggaacctcaatgttagtattccttggactcataaggtggggaactttactggtctttattcttctactgtacctgtctttaatcctcattggaaaacaccatcttttcctaatatacatttacaccaagacattatcaaaaaatgtgaacagtttgtaggcccacttacagttaatgagaaaagaagattgcaattgattatgcctgctaggttttatccaaaggttaccaaatatttaccattggataagggtattaaaccttattatccagaacatctagttaatcattacttccaaactagacactatttacacactctatggaaggcgggtatattatataagagagaaacaacacatagcgcctcattttgtgggtcaccatattcttgggaacaagatctacagcatggggcagaatctttccaccagcaatcctctgggattctttcccgaccaccagttggatccagccttcagagcaaacacagcaaatccagattgggacttcaatcccaacaaggacacctggccagacgccaacaaggtaggagctggagcattcgggctgggtttcactccaccgcacggaggccttttggggtggagctctcaggctcagggcatactacaaactttgccagcaaatccgcctcctgcctccaccaatcgccagacaggaaggcagcctaccccgctgtctccacctttgagaaacactcatcctcaggccatgcagtggaa

SEQ ID NO: 7 - DNA, 3212 bp, Hepatitis B virus
  HBV genotype E (1)..(3212)
ttccacaacattccaccaagctcascaggatcccagagtaagrggcctgtatyttcctgctggtggctccagttccggaacagtgaaccctgttccgactactgcctcactcatctcgtcaatcttctcgaggattggggaccctgcaccgaacatggaaggcatcacatcaggattcctaggacccctgctcgtgttacaggcggggtttttcttgttgacaaaaatcctcacaataccgcagagtctagactcgtggtggacttctctcaattttcyaggggaagctcccgtgtgtcgtggccaaaattcgcagtycccaacctccaatcactcaccaacctcttgtcctccaatttgtcctggctatcgctggatgtgtctgcggcgttttatcatcttcctcttcatcctgctgctatgcctcatcttcttgttggttcttctggactatcaaggtatgttgcccgtttgtcctctaattccaggatcatcaaccaccagtacgggaccctgccgaacctgcacgactcttgctcaaggaacctctatgtttccctcatgttgctgttcaaaaccttcggacggaaattgcacttgtattcccatcccatcatcatgggctttcggaaaattcctatgggagtgggcctcagcccgtttctcctggctcagtttactagtgccatttgttcagtggttcgccgggctttcccccactgtctggctttcagttatatggatgatgtggtattgggggccaagtctgtacaacatcttgagtccctttatacctctgttaccaattttcttttgtctttgggtatacatttaaatcctaacaaaacaaaaagatggggatattccctaaatttcatgggttatgttattggtagttgggggtcattaccacaggaacacatcagaatgaaaatcaaagactgttttagaaaactccctgttaaccggcctattgattggaaagtatgtcaaagaattgtgggtctcttgggctttgctgccccttttacacaatgtggatatcctgctttaatgcctctgtatgcgtgtattcaatctaagcaggctttcactttctcgccaacttacaaggcctttctgtgtaaacaatacctgaacctttaccccgttgcccggcaacggccaggtctgtgccaagtgtttgctgatgcaacccccactggttggggcttggccataggccatcagcgcatgcgtggaacctttgyggctcctctgccgatccatactgcggaactcctggccgcttgttttgctcgcagcaggtctggagcgaaacttattggaacggataattctgtcgttctctcccggaaatatacatcatttccatggctgctaggctgtgctgccaactggatcctgcgagggacgtcctttgtctacgtcccgtcagcgctgaatcctgcggacgacccgtctcggggtcgcttggggatctatcgtccccttctccgtctgccgttccggccgaccacggggcgcacctctctttacgcggtctccccgtctgtgccttctcatctgccggaccgtgtgcacttcgcttcacctctgcacgtcgcatggaaaccaccgtgaacgcccaccaaatcttgcccaaggtcttatataagaggactcttggactctctgcaatgtcaacgaccgaccttgaggcatacttcaaagactgcttgtttaaagactgggaggagttgggggaggagattagattaatgatctttgtactaggaggctgtaggcataaattggtctgcgcaccagcaccatgcaactttttcacctctgcctaatcatctcttgttcatgtcctactgttcaagcctccaagctgtgccttgggtggctttaggacatggacattgacccttataaagaatttggagctwctgtggagttactctcktttttgcctcatgacttctttccttcaataagagatcttctagataccgccacagctctgtatcgggatgccttagaatctcctgagcattgttcacctcaccacacggcactcaggcaagccattctttgctggggggatgtaatgaatctagctacctgggtgggtgtaaatttggaagatccagcatccagggacctggtagtcggttatgtcaatactaatatgggcctaaagttcagacaattattgtggtttcacacttcctgtctcacttttggaagagaaaccgtcttagagtatttggtgtcttttggagtgtggattcgcactcctccaccttatagaccaccaaatgcccctatcttatcaacacttccggagactactgttgttagacgaagaggcaggtcccctagaagaagaactccctcrcctcgcagacgtagatctcaatcgccgcgtcgcagaagatctcaatctccagcttcccgatgttagtattccttggactcacaaggtgggaaattttacggggctttactcttctactatacctgtctttaatcctaactggaaaactccatcttttcctgatattcatttgcaccaggacattattaacaaatgtgaacaatttgtaggtcccctaacagtaaatgaaaaacgaagattmaacttagtcatgcctgctagattttttcccatctctacgaaatatttgcctctagagaaaggtataaaaccctattatccagataatgtagttaatcattacttccaaaccagacactatttacataccctatggaaggcgggtatcttatataaaagagaaactgcacgtagcgcctcattttgtgggtcaccatattcttgggaacaagagctacatcatgggtctttcttggacggtccctctcgaatgggggaagaatcattccaccaccaatcctctgggattttttcccgaccaccagttggatccagcattcagagcaaacaccagaaatccagattgggaccacaatcccaacaaagaccactggacagaagccaacaaggtaggagtgggagcattcgggccggggttcactcccccacacggaggccttttggggtggagccctcaggctcaaggcatgctaaaaacattgccagcagatccgcctcctgcctccaccaatcggcagtcaggaaggcagcctaccccaatcactccacctttgagagacactcatcctcaggccatrcagtggaa

SEQ ID NO: 8 - DNA, 3205 bp, Hepatitis B virus
  HBV genotype F (1)..(3205)
ttccatcaggctctgttggatcccagggtaagggctctgtatcttcctgctggtggctccagttcaggaacacaaaaccctgctccgactattgcctctctcacatcctcaatcttctcgacgactgggggccctgctatgaacatggacaacattacatcaggactcctaggacccctgctcgtgttacaggcggtgtgtttcttgttgacaaaaatcctcacaataccacagagtctagactcgtggtggacttctctcaattttctagggggactacccgggtgtcctggccaaaattcgcagtccccaacctccaatcacttaccaacctcctgtcctccaacttgtcctggctatcgttggatgtgtctgcggcgttttatcatcttcctcttcatcctgctgctatgcctcatcttcttgttggttcttctggactaccagggtatgttgcccgtttgtcctctacttccaggatccacgaccaccagcacgggaccctgcaaaacctgcacaactcttgcacaaggaacctctatgtttccctcctgttgctgttcaaaaccctcggacggaaactgcacttgtattcccatcccatcatcctgggctttaggaaaatacctatgggagtgggcctcagcccgtttctcatggctcagtttactagtgcaatttgttcagtggtgcgtagggctttcccccactgtctggcttttagttatattgatgatctggtattgggggccaaatctgtgcagcaccttgagtccctttataccgctgttaccaattttctgttatctgtgggtatccatttaaatacttctaaaactaagagatggggttacaccctacattttatgggttatgtcattggtagttggggatcattacctcaagatcatattgtacacaaaatcaaagaatgttttcggaaactgcctgtaaatcgtccaattgattggaaagtctgtcaacgcattgtgggtcttttgggctttgctgcccctttcacacaatgtggttatcctgctctcatgcctctgtatgcttgtattactgctaaacaggcttttgttttttcgccaacttacaaggcctttctctgtaaacaatacatgaacctttaccccgttgccaggcaacggccgggcctgtgccaagtgtttgctgacgcaacccccactggttggggcttggccattggccatcagcgcatgcgtggaacctttgtggctcctctgccgatccatactgcggaactccttgcagcttgtttcgctcgcagcaggtctggagcgactctcatcggcacggacaactctgttgtcctctctaggaagtacacctccttcccatggctgctcgggtgtgctgcaaactggatcctgcgcgggacgtcctttgtttacgtcccgtcggcgctgaatcccgcggacgacccctcccggggccgcttggggctgtaccgccctcttctccgtctgccgttccagccgacaacgggtcgcacctctctttacgcggactccccgtctgttccttctcatctgccggaccgtgtgcacttcgcttcacctctgcacgtcgcatggagaccaccgtgaacgccccttggagtttgccaacagtcttacataagaggactcttggactttcaggagggtcaatgacccggattgcagaatacatcaaagactgtgtatttaaggactgggaggagttgggggaggagactaggttaatgatctttgtactaggaggctgtaggcataaattggtctgttcaccagcaccatgcaactttttcacctctgcctaatcatcttttgttcatgtcctactgttcaagcctccaagctgtgccttgggtggctttgggacatggacattgacccttataaagaatttggcgcttctgtggagttactctcttttttgccttctgatttctttccatcggttcgggacctactcgacaccgcttcagccctttaccgggatgctttagagtcacctgaacattgcactccccatcacactgccctcaggcaagttattttgtgctggggtgagttaatgactttggcttcctgggtgggcaataacttggaagaccctgctgccagggatttagtagttaactatgttaacactaacatgggcctaaaaattagacaactactgtggtttcacatttcctgccttacttttggaagagatatagttcttgagtatttggtgtcctttggagtgtggattcgcactcctcctgcttacagaccacaaaatgcccctatcctatccacacttccggaaactactgttgttagacgacgaggcaggtcccctagaagaagaactccctcgcctcgcagacgaagatctcaatcgccgcgtcgccgaagatctcaatctccagcttcccaatgttagtattccttggactcataaggtgggaaattttacggggctttactcttctactgtgcctgcttttaatcctgactggttaactccttcttttcctaatattcatttacatcaagacctaatttctaaatgtgaacaatttgtaggcccactcactaaaaatgaattaaggaggttaaaattggttatgccagctagattttatcctaaggttaccaaatattttcctatggagaaaggaatcaagccttattatcctgagcatgcagttaatcattactttaaaacaagacattatttgcatactttatggaaggcgggaattttatataagagagaatccacacgtagcgcatcattttgtgggtcaccatattcctgggaacaagagctacagcatgggagcacctctctcaacgacaagaagaggcatgggacagaatctttctgtgcccaatcctctgggattctttccagaccatcagctggatccgctattcaaagcaaattccagcagtcccgactgggacttcaacacaaacaaggacagttggccaatggcaaacaaggtaggagtgggagcatacggtccagggttcacacccccacacggtggcctgctggggtggagccctcaggcacaaggtatgttaacaaccttgccagcagatccgcctcctgcttccaccaatcggcggtccgggagaaagccaaccccagtctctccacctctaagagacactcatccacaggcaatgcagtggaa

SEQ ID NO: 9 - DNA, 3247 bp, Hepatitis B virus
  HBV genotype G (1)..(3247)
tctacagcattccaccaagctctacaaaatcccaaagtcaggggcctgtattttcctgctggtggctccagttcagggatagtgaaccctgttccgactattgcctctcacatctcgtcaatcttctccaggattggggaccctgcaccgaacatggagaacatcacatcaggattcctaggacccctgctcgtgttacaggcggggtttttcttgttgacaagaatcctcacaataccgcagaatctagactcgtggtggacttctctcaattttctagggggagtgcccgtgtgtcctggcctaaattcgcagtccccaacctccaatcactcaccaatctcctgtcctccaacttgtcctggctatcgctggatgtgtctgcggcgttttatcatattcctcttcatcctgctgctatgcctcatcttcttgttggttcttctggactatcaaggtatgttgcccgtttgtcctctgattccaggatcctcgaccaccagtacgggaccctgcaaaacctgcacgactcctgctcaaggcaactctatgtatccctcatgttgctgtacaaaaccttcggacggaaattgcacctgtattcccatcccatcatcttgggctttcgcaaaatacctatgggagtgggcctcagtccgtttctcttggctcagtttactagtgccatttgttcagtggttcgtagggctttcccccactgtctggctttcagctatatggatgatgtggtattgggggccaaatctgtacaacatcttgagtccctttataccgctgttaccaattttcttttgtctttgggtatacatctaaaccctaacaaaacaaaaagatggggttattccttaaattttatgggatatgtaattggaagttggggtactttgccacaagaacacatcacacagaaaattaagcaatgttttcggaaactccctgttaacaggccaattgattggaaagtctgtcaacgaataactggtctgttgggtttcgctgctccttttacccaatgtggttaccctgccttaatgcctttatatgcatgtatacaagctaagcaggcttttactttctcgccaacttataaggcctttctctgtaaacaatacatgaacctttaccccgttgctaggcaacggcccggtctgtgccaagtgtttgctgacgcaacccccactggttggggcttggccatcggccatcagcgcatgcgtggaacctttgtggctcctctgccgatccatactgcggaactcctagctgcttgttttgctcgcagccggtctggagcaaaactcattgggactgacaattctgtcgtcctttctcggaaatatacatcctttccatggctgctaggctgtgctgccaactggatccttcgcgggacgtcctttgtttacgtcccgtcagcgctgaatccagcggacgacccctcccggggccgtttggggctctgtcgcccccttctccgtctgccgttcctgccgaccacggggcgcacctctctttacgcggtctccccgtctgttccttctcatctgccggaccgtgtgcacttcgcttcacctctgcacgttacatggaaaccgccatgaacacctctcatcatctgccaaggcagttatataagaggactcttggactgtttgttatgtcaacaaccggggtggagaaatacttcaaggactgtgtttttgctgagtgggaagaattaggcaatgagtccaggttaatgacctttgtattaggaggctgtaggcataaattggtctgcgcaccagcaccatgtaactttttcacctctgcctaatcatctcttgttcatgtcctactgttcaagcctccaagctgtgccttgggtggctttagggcatggatagaacaactttgccatatggcctttttggcttagacattgacccttataaagaatttggagctactgtggagttgctctcgtttttgccttctgactttttcccgtctgttcgtgatcttctcgacaccgcttcagctttgtaccgggaatccttagagtcctctgatcattgttcgcctcaccatacagcactcaggcaagcaatcctgtgctggggtgagttgatgactctagccacctgggtgggtaataatttggaagatccagcatccagagatttggtggtcaattatgttaatactaatatgggtttaaaaatcaggcaactattgtggtttcacatttcctgtcttacttttgggagagaaaccgttcttgagtatttggtgtcttttggagtgtggattcgcactcctcctgcttatagaccaccaaatgcccctatcctatcaacacttccggagactactgttgttagacgaagaggcaggtcccctcgaagaagaactccctcgcctcgcagacgaagatctcaatcgccgcgtcgcagaagatctgcatctccagcttcccaatgttagtattccttggactcacaaggtgggaaactttacggggctgtattcttctactatacctgtctttaatcctgattggcaaactccttcttttccaaatatccatttgcatcaagacattataactaaatgtgaacaatttgtgggccctctcacagtaaatgagaaacgaagattaaaactagttatgcctgccagatttttcccaaactctactaaatatttaccattagacaaaggtatcaaaccgtattatccagaaaatgtagttaatcattacttccagaccagacattatttacataccctttggaaggcgggtattctatataagagagaaacatcccgtagcgcttcattttgtgggtcaccatatacttgggaacaagatctacagcatggggctttcttggacggtccctctcgagtggggaaagaacctttccaccagcaatcctctaggattccttcccgatcaccagttggacccagcattcagagcaaataccaacaatccagattgggacttcaatcccaaaaaggacccttggccagaggccaacaaggtaggagttggagcctatggacccgggttcacccctccacacggaggccttttggggtggagccctcagtctcagggcacactaacaactttgccagcagatccgcctcctgcctccaccaatcgtcagtcagggaggcagccgactcccatctctccaccactaagagacagtcatcctcaggccatgcagtggaa

SEQ ID NO: 10 - DNA, 22 bp, Hepatitis B virus
  HBV 1-2 recognition sequence (sense) (1)..(22)
cccctgctcgtgttacaggcgg

SEQ ID NO: 11 - DNA, 22 bp, Hepatitis B virus
  HBV 1-2 recognition sequence (antisense) (1)..(22)
ggggacgagcacaatgtccgcc

SEQ ID NO: 12 - DNA, 22 bp, Hepatitis B virus
  HBV 5-6 recognition sequence (sense) (1)..(22)
gatgatgtggtattgggggcca

SEQ ID NO: 13 - DNA, 22 bp, Hepatitis B virus
  HBV 5-6 recognition sequence (antisense) (1)..(22)
ctactacaccataacccccggt

SEQ ID NO: 14 - DNA, 22 bp, Hepatitis B virus
  HBV 7-8 recognition sequence (sense) (1)..(22)
tttgctgacgcaacccccactg

SEQ ID NO: 15 - DNA, 22 bp, Hepatitis B virus
  HBV 7-8 recognition sequence (antisense) (1)..(22)
aaacgactgcgttgggggtgac

SEQ ID NO: 16 - DNA, 22 bp, Hepatitis B virus
  HBV 11-12 recognition sequence (sense) (1)..(22)
tgccgatccatactgcggaact

SEQ ID NO: 17 - DNA, 22 bp, Hepatitis B virus
  HBV 11-12 recognition sequence (antisense) (1)..(22)
acggctaggtatgacgccttga

SEQ ID NO: 18 - protein, 354 aa, Artificial
  Synthetic Sequence
  HBV 1-2x.2 (1)..(354): full sequence
MNTKYNKEFLLYLAGFVDGDGSIFACIRPVQWSKFKHSLELCFTVTQKTQRRWFLDKLVDEIGVGYVHDYGSVSAYRLSQIKPLHNFLTQLQPFLKLKQKQANLVLKIIEQLPSAKESPDKFLEVCTWVDQIAALNDSKTRKTTSETVRAVLDSLPGSVGGLSPSQASSAASSASSSPGSGISEALRAGAGSGTGYNKEFLLYLAGFVDGDGSIYASIRPSQDQKFKHRLILVFAVSQKTQRRWFLDKLVDEIGVGYVRDTGSVSEYRLSEIKPLHNFLTQLQPFLKLKQKQANLVLKIIEQLPSAKESPDKFLEVCTWVDQIAALNDSKTRKTTSETVRAVLDSLSEKKKSSP

SEQ ID NO: 19 - protein, 354 aa, Artificial
  Synthetic Sequence
  HBV 1-2x.14 (1)..(354): full sequence
MNTKYNKEFLLYLAGFVDGDGSIYACIAPRQWSKFKHSLELRFAVFQKTQRRWFLDKLVDEIGVGYVSDYGSVSRYHLSEIKPLHNFLTQLQPFLKLKQKQANLVLKIIEQLPSAKESPDKFLEVCTWVDQIAALNDSKTRKTTSETVRAVLDSLPGSVGGLSPSQASSAASSASSSPGSGISEALRAGAGSGTGYNKEFLLYLAGFVDGDGSIYACIRPAQDSKFKHRLILALEVGQKTRRRWFLDKLVDEIGVGYVVDNGSVSRYILSQIKPLHNFLTQLQPFLKLKQKQANLVLKIIEQLPSAKESPDKFLEVCTWVDQIAALNDSKTRKTTSETVRAVLDSLSEKKKSSP

SEQ ID NO: 20 - protein, 354 aa, Artificial
  Synthetic Sequence
  HBV 1-2x.68 (1)..(354): full sequence
MNTKYNKEFLLYLAGFVDGDGSIYACIRPDQSSKFKHRLVLGFEVGQKTRRRWFLDKLVDEIGVGYVVDNGSVSRYILSEIKPLHNFLTQLQPFLKLKQKQANLVLKIIEQLPSAKESPDKFLEVCTWVDQIAALNDSKTRKTTSETVRAVLDSLPGSVGGLSPSQASSAASSASSSPGSGISEALRAGAGSGTGYNKEFLLYLAGFVDGDGSIYACIAPRQWSKFKHSLELRFAVFQKTQRRWFLDKLVDEIGVGYVSDYGSVSRYHLSEIKPLHNFLTQLQPFLKLKQKQANLVLKIIEQLPSAKESPDKFLEVCTWVDQIAALNDSKTRKTTSETVRAVLDSLSEKKKSSP

SEQ ID NO: 21 - protein, 354 aa, Artificial Sequence
  Synthetic Sequence
  HBV 1-2x.93 (1)..(354): full sequence
MNTKYNKEFLLYLAGFVDGDGSIYATIRPDQTYKFKHRLILQFAVSQKTQRRWFLDKLVDEIGVGYVRDTGSVSEYRLSQIKPLHNFLTQLQPFLKLKQKQANLVLKIIEQLPSAKESPDKFLEVCTWVDQIAALNDSKTRKTTSETVRAVLDSLPGSVGGLSPSQASSAASSASSSPGSGISEALRAGAGSGTGYNKEFLLYLAGFVDGDGSIFACIRPVQWSKFKHSLELCFTVTQKTQRRWFLDKLVDEIGVGYVHDYGSVSAYRLSQIKPLHNFLTQLQPFLKLKQKQANLVLKIIEQLPSAKESPDKFLEVCTWVDQIAALNDSKTRKTTSETVRAVLDSLSEKKKSSP

SEQ ID NO: 22 - protein, 354 aa, Artificial Sequence
  Synthetic Sequence
  HBV 5-6x.33 (1)..(354): full sequence
MNTKYNKEFLLYLAGFVDGDGSIYARIRPSQSSKFKHKLTLVFAVAQKTQRRWFLDKLVDEIGVGYVHDEGSVSQYRLSQIKPLHNFLTQLQPFLKLKQKQANLVLKIIEQLPSAKESPDKFLEVCTWVDQIAALNDSKTRKTTSETVRAVLDSLPGSVGGLSPSQASSAASSASSSPGSGISEALRAGAGSGTGYNKEFLLYLAGFVDGDGSIWATIEPLQKRKFKHALHLMFTVSQKTQRRWFLDKLVDEIGVGYVIDQGSVSEYRLSQIKPLHNFLTQLQPFLKLKQKQANLVLKIIEQLPSAKESPDKFLEVCTWVDQIAALNDSKTRKTTSETVRAVLDSLSEKKKSSP

SEQ ID NO: 23 - protein, 354 aa, Artificial Sequence
  Synthetic Sequence
  HBV 5-6x.84 (1)..(354): full sequence
MNTKYNKEFLLYLAGFVDGDGSIFARIRPGQDYKFKHNLVLTFRVAQKTQRRWFLDKLVDEIGVGYVLDEGSVSQYYLSEIKPLHNFLTQLQPFLKLKQKQANLVLKIIEQLPSAKESPDKFLEVCTWVDQIAALNDSKTRKTTSETVRAVLDSLPGSVGGLSPSQASSAASSASSSPGSGISEALRAGAGSGTGYNKEFLLYLAGFVDGDGSINASIEPVQKPKFKHTLHLRFEVSQKTQRRWFLDKLVDEIGVGYVYDQGSVSSYRLSEIKPLHNFLTQLQPFLKLKQKQANLVLKIIEQLPSAKESPDKFLEVCTWVDQIAALNDSKTRKTTSETVRAVLDSLSEKKKSSP

SEQ ID NO: 24 - protein, 354 aa, Artificial Sequence
  Synthetic Sequence
  HBV 5-6x.90 (1)..(354): full sequence
MNTKYNKEFLLYLAGFVDGDGSIYARIRPRQNFKFKHALVLQFRVSQKTQRRWFLDKLVDEIGVGYVLDEGSVSQYYLSQIKPLHNFLTQLQPFLKLKQKQANLVLKIIEQLPSAKESPDKFLEVCTWVDQIAALNDSKTRKTTSETVRAVLDSLPGSVGGLSPSQASSAASSASSSPGSGISEALRAGAGSGTGYNKEFLLYLAGFVDGDGSIVAQIHPAQKNKFKHGLRLQFYVYQKTQRRWFLDKLVDEIGVGYVYDQGSVSCYRLSQIKPLHNFLTQLQPFLKLKQKQANLVLKIIEQLPSAKESPDKFLEVCTWVDQIAALNDSKTRKTTSETVRAVLDSLSEKKKSSP

SEQ ID NO: 25 - protein, 354 aa, Artificial Sequence
  Synthetic Sequence
  HBV 5-6x.4 (1)..(354): full sequence
MNTKYNKEFLLYLAGFVDGDGSIYATIQPVQTRKFKHILRLWFTVHQKTQRRWFLDKLVDEIGVGYVVDAGSVSEYRLSEIKPLHNFLTQLQPFLKLKQKQANLVLKIIEQLPSAKESPDKFLEVCTWVDQIAALNDSKTRKTTSETVRAVLDSLPGSVGGLSPSQASSAASSASSSPGSGISEALRAGAGSGTGYNKEFLLYLAGFVDGDGSIYARIRPTQGSKFKHKLTLCFRVAQKTQRRWFLDKLVDEIGVGYVLDEGSVSQYYLSQIKPLHNFLTQLQPFLKLKQKQANLVLKIIEQLPSAKESPDKFLEVCTWVDQIAALNDSKTRKTTSETVRAVLDSLSEKKKSSP

SEQ ID NO: 26 - protein, 351 aa, Artificial Sequence
  Synthetic Sequence
  HBV 5-6x.5 (1)..(351): full sequence
MNTKYNKEFLLYLAGFVDGDGSIYATIHPTQKAKFKHVLALRFSVCQKTQRRWFLDKLVDEIGVGYVYDLGSVSEYRLSQIKPLHNFLTQLQPFLKLKQKQANLVLKIIEQLPSAKESPDKFLEVCTWVDQIAALNDSKTRKTTSETVRAVLDSLPGSVGGLSPSQASSAASSASSSPGSGISEALRAGAGSYNKEFLLYLAGFVDGDGSIYARIRPLQHGKFKHKLHLAFRVAQKTQRRWFLDKLVDEIGVGYVFDDGSVSQYTLSQIKPLHNFLTQLQPFLKLKQKQANLVLKIIEQLPSAKESPDKFLEVCTWVDQIAALNDSKTRKTTSETVRAVLDSLSEKKKSSP

SEQ ID NO: 27 - protein, 354 aa, Artificial Sequence
  Synthetic Sequence
  HBV 5-6x.68 (1)..(354): full sequence
MNTKYNKEFLLYLAGFVDGDGSIYAQIMPRQRAKFKHVLKLNFAVCQKTQRRWFLDKLVDEIGVGYVTDQGSVSEYRLSEIKPLHNFLTQLQPFLKLKQKQANLVLKIIEQLPSAKESPDKFLEVCTWVDQIAALNDSKTRKTTSETVRAVLDSLPGSVGGLSPSQASSAASSASSSPGSGISEALRAGAGSGTGYNKEFLLYLAGFVDGDGSIYARIRPRQSSKFKHRLLLFFRVSQKTQRRWFLDKLVDEIGVGYVLDEGSVSQYYLSEIKPLHNFLTQLQPFLKLKQKQANLVLKIIEQLPSAKESPDKFLEVCTWVDQIAALNDSKTRKTTSETVRAVLDSLSEKKKSSP

SEQ ID NO: 28 - protein, 354 aa, Artificial Sequence
  Synthetic Sequence
  HBV 5-6x.79 (1)..(354): full sequence
MNTKYNKEFLLYLAGFVDGDGSIYATIEPVQKNKFKHQLRLCFAVCQKTQRRWFLDKLVDEIGVGYVCDTGSVSEYRLSQIKPLHNFLTQLQPFLKLKQKQANLVLKIIEQLPSAKESPDKFLEVCTWVDQIAALNDSKTRKTTSETVRAVLDSLPGSVGGLSPSQASSAASSASSSPGSGISEALRAGAGSGTGYNKEFLLYLAGFVDGDGSIYARIRPCQGCKFKHALKLTFRVAQKTQRRWFLDKLVDEIGVGYVCDEGSVSQYYLSQIKPLHNFLTQLQPFLKLKQKQANLVLKIIEQLPSAKESPDKFLEVCTWVDQIAALNDSKTRKTTSETVRAVLDSLSEKKKSSP

SEQ ID NO: 29 - protein, 354 aa, Artificial Sequence
  Synthetic Sequence
  HBV 7-8x.2 (1)..(354): full sequence
MNTKYNKEFLLYLAGFVDGDGSIYATISPAQAYKFKHRLGLFFEVDQKTQRRWFLDKLVDEIGVGYVHDRGSVSRYKLSEIKPLHNFLTQLQPFLKLKQKQANLVLKIIEQLPSAKESPDKFLEVCTWVDQIAALNDSKTRKTTSETVRAVLDSLPGSVGGLSPSQASSAASSASSSPGSGISEALRAGAGSGTGYNKEFLLYLAGFVDGDGSIYARIVPCQRSKFKHALRLEFTVRQKTRRRWILDKLVDEIGVGYVYDSGSVSRYYLSQIKPLHNFLTQLQPFLKLKQKQANLVLKIIEQLPSAKESPDKFLEVCTWVDQIAALNDSKTRKTTSETVRAVLDSLSEKKKSSP

SEQ ID NO: 30 - protein, 354 aa, Artificial Sequence
  Synthetic Sequence
  HBV 7-8x.9 (1)..(354): full sequence
MNTKYNKEFLLYLAGFVDGDGSIYATISPAQAYKFKHRLGLFFEVDQKTQRRWFLDKLVDEIGVGYVHDRGSVSRYKLSQIKPLHNFLTQLQPFLKLKQKQANLVLKIIEQLPSAKESPDKFLEVCTWVDQIAALNDSKTRKTTSETVRAVLDSLPGSVGGLSPSQASSAASSASSSPGSGISEALRAGAGSGTGYNKEFLLYLAGFVDGDGSIYARIVPCQRSKFKHALRLEFTVRQKTRRRWILDKLVDEIGVGYVFDDGSVSRYYLSQIKPLHNFLTQLQPFLKLKQKQANLVLKIIEQLPSAKESPDKFLEVCTWVDQIAALNDSKTRKTTSETVRAVLDSLSEKKKSSP

SEQ ID NO: 31 - protein, 354 aa, Artificial Sequence
  Synthetic Sequence
  HBV 7-8x.17 (1)..(354): full sequence
MNTKYNKEFLLYLAGFVDGDGSIYATISPAQAYKFKHRLGLFFEVDQKTQRRWFLDKLVDEIGVGYVHDRGSVSRYKLSQIKPLHNFLTQLQPFLKLKQKQANLVLKIIEQLPSAKESPDKFLEVCTWVDQIAALNDSKTRKTTSETVRAVLDSLPGSVGGLSPSQASSAASSASSSPGSGISEALRAGAGSGTGYNKEFLLYLAGFVDGDGSIYARIVPCQRSKFKHALRLEFTVRQKTRRRWILDKLVDEIGVGYVFDDGSVSRYYLSQIKPLHNFLTQLQPFLKLKQKQANLVLKIIEQLPSAKESPDKFLEVCTWVDQIAALNDSKTRKTTSETVRAVLDRLSEKKKSSP

SEQ ID NO: 32 - protein, 354 aa, Artificial Sequence
  Synthetic Sequence
  HBV 7-8x.44 (1)..(354): full sequence
MNTKYNKEFLLYLAGFVDGDGSIYATISPAQAYKFKHRLGLFFEVDQKTQRRWFLDKLVDEIGVGYVHDRGSVSRYKLSQIKPLHNFLTQLQPFLKLKQKQANLVLKIIEQLPSAKESPDKFLEVCTWVDQIAALNDSKTRKTTSETVRAVLDSLPGSVGGLSPSQASSAASSASSSPGSGISEALRAGAGSGTGYNKEFLLYLAGFVDGDGSIYARIVPCQRSKFKHALRLEFAVRQKTQRRWILDKLVDEIGVGYVFDDGSVSRYYLSEIKPLHNFLTQLQPFLKLKQKQANLVLKIIEQLPSAKESPDKFLEVCTWVDQIAALNDSKTRKTTSETVRAVLDSLSEKKKSSP

SEQ ID NO: 33 - protein, 354 aa, Artificial Sequence
  Synthetic Sequence
  HBV 11-12x.26 (1)..(354): full sequence
MNTKYNKEFLLYLAGFVDGDGSINASIAPRQSFKFKHGLKLRFEVGQKTQRRWFLDKLVDEIGVGYVYDNGSVSVYSLSQIKPLHNFLTQLQPFLKLKQKQANLVLKIIEQLPSAKESPDKFLEVCTWVDQIAALNDSKTRKTTSETVRAVLDSLPGSVGGLSPSQASSAASSASSSPGSGISEALRAGAGSGTGYNKEFLLYLAGFVDGDGSIYASIRPRQYAKFKHDLELRFNVRQKTQRRWFLDKLVDEIGVGYVVDWGSVSTYQLSQIKPLHNFLTQLQPFLKLKQKQANLVLKIIEQLPSAKESPDKFLEVCTWVDQIAALNDSKTRKTTSETVRAVLDSLSEKKKSSP

SEQ ID NO: 34 - protein, 354 aa, Artificial Sequence
  Synthetic Sequence
  HBV 11-12x.9 (1)..(354): full sequence
MNTKYNKEFLLYLAGFVDGDGSIHACIRPRQTAKFKHSLLLRFQVGQKTQRRWFLDKLVDEIGVGYVYDNGSVSVYELSQIKPLHNFLTQLQPFLKLKQKQANLVLKIIEQLPSAKESPDKFLEVCTWVDQIAALNDSKTRKTTSETVRAVLDSLPGSVGGLSPSQASSAASSASSSPGSGISEALRAGAGSGTGYNKEFLLYLAGFVDGDGSIYAAIRPKQTRKFKHELQLTFNVRQKSQRRWFLDKLVDEIGVGYVLDWGSVSTYILSQIKPLHNFLTQLQPFLKLKQKQANLVLKIIEQLPSAKESPDKFLEVCTWVDQIAALNDSKTRKTTSETVRAVLDSLSEKKKSSP

SEQ ID NO: 35 - protein, 354 aa, Artificial Sequence
  Synthetic Sequence
  HBV 11-12x.13 (1)..(354): full sequence
MNTKYNKEFLLYLAGFVDGDGSIHACIRPRQTAKFKHSLLLRFQVGQKTQRRWFLDKLVDEIGVGYVYDNGSVSVYELSQIKPLHNFLTQLQPFLKLKQKQANLVLKIIEQLPSAKESPDKFLEVCTWVDQIAALNDSKTRKTTSETVRAVLDSLPGSVGGLSPSQASSAASSASSSPGSGISEALRAGAGSGTGYNKEFLLYLAGFVDGDGSIYAAIRPKQTRKFKHELQLTFNVRQKTQRRWFLDKLVDEIGVGYVLDWGSVSTYILSQIKPLHNFLTQLQPFLKLKQKQANLVLKIIEQLPSAKESPDKFLEVCTWVDQIAALNDSKTRKTTSETVRAVLDSLSEKKKSSP

SEQ ID NO: 36 - protein, 354 aa, Artificial Sequence
  Synthetic Sequence
  HBV 11-12x.16 (1)..(354): full sequence
MNTKYNKEFLLYLAGFVDGDGSIHATISPRQTFKFKHGLRLRFEVGQKTQRRWFLDKLVDEIGGGYVYDNGSVSVYSLSQIKPLHNFLTQLQPFLKLKQKQANLVLKIIEQLPSAKESPDKFLEVCTWVDQIAALNDSKTRKTTSETVRAVLDSLPGSVGGLSPSQASSAASSASSSPGSGISEALRAGAGSGTGYNKEFLLYLAGFVDGDGSIYASIRPRQQAKFKHSLELHFNVRQKTQRRWFLDKLVDEIGVGYVVDEGSVSTYLLSEIKPLHNFLTQLQPFLKLKQKQANLVLKIIEQLPSAKESPDKFLEVCTWVDQIAALNDSKTRKTTSETVRAVLDSLSEKKKSSP

SEQ ID NO: 37 - protein, 354 aa, Artificial Sequence
  Synthetic Sequence
  HBV 11-12x.27 (1)..(354): full sequence
MNTKYNKEFLLYLAGFVDGDGSIHACIRPRQTAKFKHSLLLRFQVGQKTQRRWFLDKLVDEIGVGYVYDNGSVSVYELSEIKPLHNFLTQLQPFLKLKQKQANLVLKIIEQLPSAKESPDKFLEVCTWVDQIAALNDSKTRKTTSETVRAVLDSLPGSVGGLSPSQASSAASSASSSPGSGISEALRAGAGSGTGYNKEFLLYLAGFVDGDGSIYASIRPRQYAKFKHDLELRFNVRQKTQRRWFLDKLVDEIGVGYVVDWGSVSTYQLSQIKPLHNFLTQLQPFLKLKQKQANLVLKIIEQLPSAKESPDKFLEVCTWVDQIAALNDSKTRKTTSETVRAVLDSLSEKKKSSP

SEQ ID NO: 38 - protein, 354 aa, Artificial Sequence
  Synthetic Sequence
  HBV 11-12x.41 (1)..(354): full sequence
MNTKYNKEFLLYLAGFVDGDGSIHACIRPRQTAKFKHSLLLRFQVGQKTQRRWFLDKLVDEIGVGYVYDNGSVSVYELSKIKPLHNFLTQLQPFLKLKQKQANLVLKIIEQLPSAKESPDKFLEVCTWVDQIAALNDSKTRKTTSETVRAVLDSLPGSVGGLSPSQASSAASSASSSPGSGISEALRAGAGSGTGYNKEFLLYLAGFVDGDGSIYASIRPRQLAKFKHTLELHFNVRQKTQRRWFLDKLVDEIGVGYVLDSGSVSTYLLSQIKPLHNFLTQLQPFLKLKQKQANLVLKIIEQLPSAKESPDKFLEVCTWVDQIAALNDSKTRKTTSETVRAVLDSLSEKKKSSP

SEQ ID NO: 39 - protein, 354 aa, Artificial Sequence
  Synthetic Sequence
  HBV 11-12x.48 (1)..(354): full sequence
MNTKYNKEFLLYLAGFVDGDGSIHACIRPRQTAKFKHSLLLRFQVGQKTQRRWFLDKLVDEIGVGYVYDNGSVSVYELSKIKPLHNFLTQLQPFLKLKQKQANLVLKIIEQLPSAKESPDKFLEVCTWVDQIAALNDSKTRKTTSETVRAVLDSLPGSVGGLSPSQASSAASSASSSPGSGISEALRAGAGSGTGYNKEFLLYLAGFVDGDGSIYAAIRPKQTRKFKHELQLTFNVRQKTQRRWFLDKLVDEIGVGYVLDWGSVSTYILSQIKPLHNFLTQLQPFLKLKQKQANLVLKIIEQLPSAKESPDKFLEVCTWVDQIAALNDSKTRKTTSETVRAVLDSLSEKKKSSP

SEQ ID NO: 40 - protein, 147 aa, Artificial Sequence
  Synthetic Sequence
  HBV 1-2x.2-2 (1)..(147): HBV1-binding subunit
KEFLLYLAGFVDGDGSIFACIRPVQWSKFKHSLELCFTVTQKTQRRWFLDKLVDEIGVGYVHDYGSVSAYRLSQIKPLHNFLTQLQPFLKLKQKQANLVLKIIEQLPSAKESPDKFLEVCTWVDQIAALNDSKTRKTTSETVRAVLD

SEQ ID NO: 41 - protein, 147 aa, Artificial Sequence
  Synthetic Sequence
  HBV 1-2x.14-2 (1)..(147): HBV1-binding subunit
KEFLLYLAGFVDGDGSIYACIAPRQWSKFKHSLELRFAVFQKTQRRWFLDKLVDEIGVGYVSDYGSVSRYHLSEIKPLHNFLTQLQPFLKLKQKQANLVLKIIEQLPSAKESPDKFLEVCTWVDQIAALNDSKTRKTTSETVRAVLD

SEQ ID NO: 42 - protein, 147 aa, Artificial Sequence; identical to SEQ ID NO: 41
  Synthetic Sequence
  HBV 1-2x.68-2 (1)..(147): HBV1-binding subunit

SEQ ID NO: 43 - protein, 147 aa, Artificial Sequence; identical to SEQ ID NO: 40
  Synthetic Sequence
  HBV 1-2x.93-2 (1)..(147): HBV1-binding subunit

SEQ ID NO: 44 - protein, 147 aa, Artificial Sequence
  Synthetic Sequence
  HBV 1-2x.2-3 (1)..(147): HBV2-binding subunit
KEFLLYLAGFVDGDGSIYASIRPSQDQKFKHRLILVFAVSQKTQRRWFLDKLVDEIGVGYVRDTGSVSEYRLSEIKPLHNFLTQLQPFLKLKQKQANLVLKIIEQLPSAKESPDKFLEVCTWVDQIAALNDSKTRKTTSETVRAVLD

SEQ ID NO: 45 - protein, 147 aa, Artificial Sequence
  Synthetic Sequence
  HBV 1-2x.14-3 (1)..(147): HBV2-binding subunit
KEFLLYLAGFVDGDGSIYACIRPAQDSKFKHRLILALEVGQKTRRRWFLDKLVDEIGVGYVVDNGSVSRYILSQIKPLHNFLTQLQPFLKLKQKQANLVLKIIEQLPSAKESPDKFLEVCTWVDQIAALNDSKTRKTTSETVRAVLD

SEQ ID NO: 46 - protein, 147 aa, Artificial Sequence
  Synthetic Sequence
  HBV 1-2x.68-3 (1)..(147): HBV2-binding subunit
KEFLLYLAGFVDGDGSIYACIRPDQSSKFKHRLVLGFEVGQKTRRRWFLDKLVDEIGVGYVVDNGSVSRYILSEIKPLHNFLTQLQPFLKLKQKQANLVLKIIEQLPSAKESPDKFLEVCTWVDQIAALNDSKTRKTTSETVRAVLD

SEQ ID NO: 47 - protein, 147 aa, Artificial Sequence
  Synthetic Sequence
  HBV 1-2x.93-3 (1)..(147): HBV2-binding subunit
KEFLLYLAGFVDGDGSIYATIRPDQTYKFKHRLILQFAVSQKTQRRWFLDKLVDEIGVGYVRDTGSVSEYRLSQIKPLHNFLTQLQPFLKLKQKQANLVLKIIEQLPSAKESPDKFLEVCTWVDQIAALNDSKTRKTTSETVRAVLD

SEQ ID NO: 48 - protein, 147 aa, Artificial Sequence
  Synthetic Sequence
  HBV 5-6x.33-2 (1)..(147): HBV5-binding subunit
KEFLLYLAGFVDGDGSIWATIEPLQKRKFKHALHLMFTVSQKTQRRWFLDKLVDEIGVGYVIDQGSVSEYRLSQIKPLHNFLTQLQPFLKLKQKQANLVLKIIEQLPSAKESPDKFLEVCTWVDQIAALNDSKTRKTTSETVRAVLD

SEQ ID NO: 49 - protein, 147 aa, Artificial Sequence
  Synthetic Sequence
  HBV 5-6x.84-2 (1)..(147): HBV5-binding subunit
KEFLLYLAGFVDGDGSINASIEPVQKPKFKHTLHLRFEVSQKTQRRWFLDKLVDEIGVGYVYDQGSVSSYRLSEIKPLHNFLTQLQPFLKLKQKQANLVLKIIEQLPSAKESPDKFLEVCTWVDQIAALNDSKTRKTTSETVRAVLD

SEQ ID NO: 50 - protein, 147 aa, Artificial Sequence
  Synthetic Sequence
  HBV 5-6x.90-2 (1)..(147): HBV5-binding subunit
KEFLLYLAGFVDGDGSIVAQIHPAQKNKFKHGLRLQFYVYQKTQRRWFLDKLVDEIGVGYVYDQGSVSCYRLSQIKPLHNFLTQLQPFLKLKQKQANLVLKIIEQLPSAKESPDKFLEVCTWVDQIAALNDSKTRKTTSETVRAVLD

SEQ ID NO: 51 - protein, 147 aa, Artificial Sequence
  Synthetic Sequence
  HBV 5-6x.4-2 (1)..(147): HBV5-binding subunit
KEFLLYLAGFVDGDGSIYATIQPVQTRKFKHILRLWFTVHQKTQRRWFLDKLVDEIGVGYVVDAGSVSEYRLSEIKPLHNFLTQLQPFLKLKQKQANLVLKIIEQLPSAKESPDKFLEVCTWVDQIAALNDSKTRKTTSETVRAVLD

SEQ ID NO: 52 - protein, 147 aa, Artificial Sequence
  Synthetic Sequence
  HBV 5-6x.5-2 (1)..(147): HBV5-binding subunit
KEFLLYLAGFVDGDGSIYATIHPTQKAKFKHVLALRFSVCQKTQRRWFLDKLVDEIGVGYVYDLGSVSEYRLSQIKPLHNFLTQLQPFLKLKQKQANLVLKIIEQLPSAKESPDKFLEVCTWVDQIAALNDSKTRKTTSETVRAVLD

SEQ ID NO: 53 - protein, 147 aa, Artificial Sequence
  Synthetic Sequence
  HBV 5-6x.68-2 (1)..(147): HBV5-binding subunit
KEFLLYLAGFVDGDGSIYAQIMPRQRAKFKHVLKLNFAVCQKTQRRWFLDKLVDEIGVGYVTDQGSVSEYRLSEIKPLHNFLTQLQPFLKLKQKQANLVLKIIEQLPSAKESPDKFLEVCTWVDQIAALNDSKTRKTTSETVRAVLD

SEQ ID NO: 54 - protein, 147 aa, Artificial Sequence
  Synthetic Sequence
  HBV 5-6x.79-2 (1)..(147): HBV5-binding subunit
KEFLLYLAGFVDGDGSIYATIEPVQKNKFKHQLRLCFAVCQKTQRRWFLDKLVDEIGVGYVCDTGSVSEYRLSQIKPLHNFLTQLQPFLKLKQKQANLVLKIIEQLPSAKESPDKFLEVCTWVDQIAALNDSKTRKTTSETVRAVLD

SEQ ID NO: 55 - protein, 147 aa, Artificial Sequence
  Synthetic Sequence
  HBV 5-6x.33-3 (1)..(147): HBV6-binding subunit
KEFLLYLAGFVDGDGSIYARIRPSQSSKFKHKLTLVFAVAQKTQRRWFLDKLVDEIGVGYVHDEGSVSQYRLSQIKPLHNFLTQLQPFLKLKQKQANLVLKIIEQLPSAKESPDKFLEVCTWVDQIAALNDSKTRKTTSETVRAVLD

SEQ ID NO: 56 - protein, 147 aa, Artificial Sequence
  Synthetic Sequence
  HBV 5-6x.84-3 (1)..(147): HBV6-binding subunit
KEFLLYLAGFVDGDGSIFARIRPGQDYKFKHNLVLTFRVAQKTQRRWFLDKLVDEIGVGYVLDEGSVSQYYLSEIKPLHNFLTQLQPFLKLKQKQANLVLKIIEQLPSAKESPDKFLEVCTWVDQIAALNDSKTRKTTSETVRAVLD

SEQ ID NO: 57 - protein, 147 aa, Artificial Sequence
  Synthetic Sequence
  HBV 5-6x.90-3 (1)..(147): HBV6-binding subunit
KEFLLYLAGFVDGDGSIYARIRPRQNFKFKHALVLQFRVSQKTQRRWFLDKLVDEIGVGYVLDEGSVSQYYLSQIKPLHNFLTQLQPFLKLKQKQANLVLKIIEQLPSAKESPDKFLEVCTWVDQIAALNDSKTRKTTSETVRAVLD

SEQ ID NO: 58 - protein, 147 aa, Artificial Sequence
  Synthetic Sequence
  HBV 5-6x.4-3 (1)..(147): HBV6-binding subunit
KEFLLYLAGFVDGDGSIYARIRPTQGSKFKHKLTLCFRVAQKTQRRWFLDKLVDEIGVGYVLDEGSVSQYYLSQIKPLHNFLTQLQPFLKLKQKQANLVLKIIEQLPSAKESPDKFLEVCTWVDQIAALNDSKTRKTTSETVRAVLD

SEQ ID NO: 59 - protein, 147 aa, Artificial Sequence
  Synthetic Sequence
  HBV 5-6x.5-3 (1)..(147): HBV6-binding subunit
KEFLLYLAGFVDGDGSIYARIRPLQHGKFKHKLHLAFRVAQKTQRRWFLDKLVDEIGVGYVFDDGSVSQYTLSQIKPLHNFLTQLQPFLKLKQKQANLVLKIIEQLPSAKESPDKFLEVCTWVDQIAALNDSKTRKTTSETVRAVLD

SEQ ID NO: 60 - protein, 147 aa, Artificial Sequence
  Synthetic Sequence
  HBV 5-6x.68-3 (1)..(147): HBV6-binding subunit
KEFLLYLAGFVDGDGSIYARIRPRQSSKFKHRLLLFFRVSQKTQRRWFLDKLVDEIGVGYVLDEGSVSQYYLSEIKPLHNFLTQLQPFLKLKQKQANLVLKIIEQLPSAKESPDKFLEVCTWVDQIAALNDSKTRKTTSETVRAVLD

SEQ ID NO: 61 - protein, 147 aa, Artificial Sequence
  Synthetic Sequence
  HBV 5-6x.79-3 (1)..(147): HBV6-binding subunit
KEFLLYLAGFVDGDGSIYARIRPCQGCKFKHALKLTFRVAQKTQRRWFLDKLVDEIGVGYVCDEGSVSQYYLSQIKPLHNFLTQLQPFLKLKQKQANLVLKIIEQLPSAKESPDKFLEVCTWVDQIAALNDSKTRKTTSETVRAVLD

SEQ ID NO: 62 - protein, 147 aa, Artificial Sequence
  Synthetic Sequence
  HBV 7-8x.2-2 (1)..(147): HBV7-binding subunit
KEFLLYLAGFVDGDGSIYARIVPCQRSKFKHALRLEFTVRQKTRRRWILDKLVDEIGVGYVYDSGSVSRYYLSQIKPLHNFLTQLQPFLKLKQKQANLVLKIIEQLPSAKESPDKFLEVCTWVDQIAALNDSKTRKTTSETVRAVLD

SEQ ID NO: 63 - protein, 147 aa, Artificial Sequence
  Synthetic Sequence
  HBV 7-8x.9-2 (1)..(147): HBV7-binding subunit
KEFLLYLAGFVDGDGSIYARIVPCQRSKFKHALRLEFTVRQKTRRRWILDKLVDEIGVGYVFDDGSVSRYYLSQIKPLHNFLTQLQPFLKLKQKQANLVLKIIEQLPSAKESPDKFLEVCTWVDQIAALNDSKTRKTTSETVRAVLD

SEQ ID NO: 64 - protein, 147 aa, Artificial Sequence; identical to SEQ ID NO: 63
  Synthetic Sequence
  HBV 7-8x.17-2 (1)..(147)

SEQ ID NO: 65 - protein, 147 aa, Artificial Sequence
  Synthetic Sequence
  HBV 7-8x.44-2 (1)..(147): HBV7-binding subunit
KEFLLYLAGFVDGDGSIYARIVPCQRSKFKHALRLEFAVRQKTQRRWILDKLVDEIGVGYVFDDGSVSRYYLSEIKPLHNFLTQLQPFLKLKQKQANLVLKIIEQLPSAKESPDKFLEVCTWVDQIAALNDSKTRKTTSETVRAVLD

SEQ ID NO: 66 - protein, 147 aa, Artificial Sequence
  Synthetic Sequence
  HBV 7-8x.2-3 (1)..(147): HBV8-binding subunit
KEFLLYLAGFVDGDGSIYATISPAQAYKFKHRLGLFFEVDQKTQRRWFLDKLVDEIGVGYVHDRGSVSRYKLSEIKPLHNFLTQLQPFLKLKQKQANLVLKIIEQLPSAKESPDKFLEVCTWVDQIAALNDSKTRKTTSETVRAVLD

SEQ ID NO: 67 - protein, 147 aa, Artificial Sequence
  Synthetic Sequence
  HBV 7-8x.9-3 (1)..(147): HBV8-binding subunit
KEFLLYLAGFVDGDGSIYATISPAQAYKFKHRLGLFFEVDQKTQRRWFLDKLVDEIGVGYVHDRGSVSRYKLSQIKPLHNFLTQLQPFLKLKQKQANLVLKIIEQLPSAKESPDKFLEVCTWVDQIAALNDSKTRKTTSETVRAVLD

SEQ ID NO: 68 - protein, 147 aa, Artificial Sequence; identical to SEQ ID NO: 67
  Synthetic Sequence
  HBV 7-8x.17-3 (1)..(147): HBV8-binding subunit

SEQ ID NO: 69 - protein, 147 aa, Artificial Sequence; identical to SEQ ID NO: 67
  Synthetic Sequence
  HBV 7-8x.44-3 (1)..(147): HBV8-binding subunit

SEQ ID NO: 70 - protein, 147 aa, Artificial Sequence
  Synthetic Sequence
  HBV 11-12x.26-2 (1)..(147): HBV11-binding subunit
KEFLLYLAGFVDGDGSIYASIRPRQYAKFKHDLELRFNVRQKTQRRWFLDKLVDEIGVGYVVDWGSVSTYQLSQIKPLHNFLTQLQPFLKLKQKQANLVLKIIEQLPSAKESPDKFLEVCTWVDQIAALNDSKTRKTTSETVRAVLD

SEQ ID NO: 71 - protein, 147 aa, Artificial Sequence
  Synthetic Sequence
  HBV 11-12x.9-2 (1)..(147): HBV11-binding subunit
KEFLLYLAGFVDGDGSIYAAIRPKQTRKFKHELQLTFNVRQKSQRRWFLDKLVDEIGVGYVLDWGSVSTYILSQIKPLHNFLTQLQPFLKLKQKQANLVLKIIEQLPSAKESPDKFLEVCTWVDQIAALNDSKTRKTTSETVRAVLD

SEQ ID NO: 72 - protein, 147 aa, Artificial Sequence
  Synthetic Sequence
  HBV 11-12x.13-2 (1)..(147): HBV11-binding subunit
KEFLLYLAGFVDGDGSIYAAIRPKQTRKFKHELQLTFNVRQKTQRRWFLDKLVDEIGVGYVLDWGSVSTYILSQIKPLHNFLTQLQPFLKLKQKQANLVLKIIEQLPSAKESPDKFLEVCTWVDQIAALNDSKTRKTTSETVRAVLD

SEQ ID NO: 73 - protein, 147 aa, Artificial Sequence
  Synthetic Sequence
  HBV 11-12x.16-2 (1)..(147): HBV11-binding subunit
KEFLLYLAGFVDGDGSIYASIRPRQQAKFKHSLELHFNVRQKTQRRWFLDKLVDEIGVGYVVDEGSVSTYLLSEIKPLHNFLTQLQPFLKLKQKQANLVLKIIEQLPSAKESPDKFLEVCTWVDQIAALNDSKTRKTTSETVRAVLD

SEQ ID NO: 74 - protein, 147 aa, Artificial Sequence; identical to SEQ ID NO: 70
  Synthetic Sequence
  HBV 11-12x.27-2 (1)..(147): HBV11-binding subunit

SEQ ID NO: 75 - protein, 147 aa, Artificial Sequence
  Synthetic Sequence
  HBV 11-12x.41-2 (1)..(147): HBV11-binding subunit
KEFLLYLAGFVDGDGSIYASIRPRQLAKFKHTLELHFNVRQKTQRRWFLDKLVDEIGVGYVLDSGSVSTYLLSQIKPLHNFLTQLQPFLKLKQKQANLVLKIIEQLPSAKESPDKFLEVCTWVDQIAALNDSKTRKTTSETVRAVLD

SEQ ID NO: 76 - protein, 147 aa, Artificial Sequence; identical to SEQ ID NO: 72
  Synthetic Sequence
  HBV 11-12x.48-2 (1)..(147): HBV11-binding subunit

SEQ ID NO: 77 - protein, 147 aa, Artificial Sequence
  Synthetic Sequence
  HBV 11-12x.26-3 (1)..(147): HBV12-binding subunit
KEFLLYLAGFVDGDGSINASIAPRQSFKFKHGLKLRFEVGQKTQRRWFLDKLVDEIGVGYVYDNGSVSVYSLSQIKPLHNFLTQLQPFLKLKQKQANLVLKIIEQLPSAKESPDKFLEVCTWVDQIAALNDSKTRKTTSETVRAVLD

SEQ ID NO: 78 - protein, 147 aa, Artificial Sequence
  Synthetic Sequence
  HBV 11-12x.9-3 (1)..(147): HBV12-binding subunit
KEFLLYLAGFVDGDGSIHACIRPRQTAKFKHSLLLRFQVGQKTQRRWFLDKLVDEIGVGYVYDNGSVSVYELSQIKPLHNFLTQLQPFLKLKQKQANLVLKIIEQLPSAKESPDKFLEVCTWVDQIAALNDSKTRKTTSETVRAVLD

SEQ ID NO: 79 - protein, 147 aa, Artificial Sequence; identical to SEQ ID NO: 78
  Synthetic Sequence
  HBV 11-12x.13-3 (1)..(147): HBV12-binding subunit

SEQ ID NO: 80 - protein, 147 aa, Artificial Sequence
  Synthetic Sequence
  HBV 11-12x.16-3 (1)..(147): HBV12-binding subunit
KEFLLYLAGFVDGDGSIHATISPRQTFKFKHGLRLRFEVGQKTQRRWFLDKLVDEIGGGYVYDNGSVSVYSLSQIKPLHNFLTQLQPFLKLKQKQANLVLKIIEQLPSAKESPDKFLEVCTWVDQIAALNDSKTRKTTSETVRAVLD

SEQ ID NO: 81 - protein, 147 aa, Artificial Sequence
  Synthetic Sequence
  HBV 11-12x.27-3 (1)..(147): HBV12-binding subunit
KEFLLYLAGFVDGDGSIHACIRPRQTAKFKHSLLLRFQVGQKTQRRWFLDKLVDEIGVGYVYDNGSVSVYELSEIKPLHNFLTQLQPFLKLKQKQANLVLKIIEQLPSAKESPDKFLEVCTWVDQIAALNDSKTRKTTSETVRAVLD

SEQ ID NO: 82 - protein, 147 aa, Artificial Sequence
  Synthetic Sequence
  HBV 11-12x.41-3 (1)..(147): HBV12-binding subunit
KEFLLYLAGFVDGDGSIHACIRPRQTAKFKHSLLLRFQVGQKTQRRWFLDKLVDEIGVGYVYDNGSVSVYELSKIKPLHNFLTQLQPFLKLKQKQANLVLKIIEQLPSAKESPDKFLEVCTWVDQIAALNDSKTRKTTSETVRAVLD

SEQ ID NO: 83 - protein, 147 aa, Artificial Sequence; identical to SEQ ID NO: 82
  Synthetic Sequence
  HBV 11-12x.48-3 (1)..(147): HBV12-binding subunit

SEQ ID NO: 84 - DNA, 22 bp, Hepatitis B virus
ccccttctcgtgttacaggcgg

SEQ ID NO: 85 - DNA, 22 bp, Hepatitis B virus
gatgatctggtattgggggcca

SEQ ID NO: 86 - DNA, 22 bp, Hepatitis B virus
tttgctgatgcaacccccactg